European Patent Application EP 4 570 910 A1, published June 18, 2025. Title: Anti-FGF23 antibodies or antibody fragments thereof. Applicant: 協和キリン株式会社. The sequence listing filed with the application follows.

SEQUENCE LISTING (59 sequences)

SEQ ID NO: 1 - protein, 117 aa, synthetic construct
  REGION 1..117: note = description of the artificial sequence: the amino acid sequenceof A antibody VH
QVQLVQSGAEVKKPGASVKVSCKASGYTFTNHYMHWVRQAPGQGLEWMGIINPISGSTSNAQKFQGRVTMTRDTSTSTVYMELSSLRSEDTAVYYCARDIVDAFDFWGQGTMVTVSS

SEQ ID NO: 2 - protein, 106 aa, synthetic construct
  REGION 1..106: note = description of the artificial sequence: the amino acid sequenceof A antibody VL
AIQLTQSPSSLSASVGDRVTITCRASQGISSALVWYQQKPGKAPKLLIYDASSLESGVPSRFSGSGSGTDFTLTISSLQPEDFATYYCQQFNDYFTFGPGTKVDIK

SEQ ID NO: 3 - protein, 117 aa, synthetic construct
  REGION 1..117: note = description of the artificial sequence: the amino acid sequenceof I100A antibody VH
QVQLVQSGAEVKKPGASVKVSCKASGYTFTNHYMHWVRQAPGQGLEWMGIINPISGSTSNAQKFQGRVTMTRDTSTSTVYMELSSLRSEDTAVYYCARDAVDAFDFWGQGTMVTVSS

SEQ ID NO: 4 - protein, 117 aa, synthetic construct
  REGION 1..117: note = description of the artificial sequence: the amino acid sequenceof I100L antibody VH
QVQLVQSGAEVKKPGASVKVSCKASGYTFTNHYMHWVRQAPGQGLEWMGIINPISGSTSNAQKFQGRVTMTRDTSTSTVYMELSSLRSEDTAVYYCARDLVDAFDFWGQGTMVTVSS

SEQ ID NO: 5 - protein, 117 aa, synthetic construct
  REGION 1..117: note = description of the artificial sequence: the amino acid sequenceof I100V antibody VH
QVQLVQSGAEVKKPGASVKVSCKASGYTFTNHYMHWVRQAPGQGLEWMGIINPISGSTSNAQKFQGRVTMTRDTSTSTVYMELSSLRSEDTAVYYCARDVVDAFDFWGQGTMVTVSS

SEQ ID NO: 6 - protein, 117 aa, synthetic construct
  REGION 1..117: note = description of the artificial sequence: the amino acid sequenceof I100Y antibody VH
QVQLVQSGAEVKKPGASVKVSCKASGYTFTNHYMHWVRQAPGQGLEWMGIINPISGSTSNAQKFQGRVTMTRDTSTSTVYMELSSLRSEDTAVYYCARDYVDAFDFWGQGTMVTVSS

SEQ ID NO: 7 - protein, 117 aa, synthetic construct
  REGION 1..117: note = description of the artificial sequence: the amino acid sequenceof I100W antibody VH
QVQLVQSGAEVKKPGASVKVSCKASGYTFTNHYMHWVRQAPGQGLEWMGIINPISGSTSNAQKFQGRVTMTRDTSTSTVYMELSSLRSEDTAVYYCARDWVDAFDFWGQGTMVTVSS

SEQ ID NO: 8 - protein, 117 aa, synthetic construct
  REGION 1..117: note = description of the artificial sequence: the amino acid sequenceof I100T antibody VH
QVQLVQSGAEVKKPGASVKVSCKASGYTFTNHYMHWVRQAPGQGLEWMGIINPISGSTSNAQKFQGRVTMTRDTSTSTVYMELSSLRSEDTAVYYCARDTVDAFDFWGQGTMVTVSS

SEQ ID NO: 9 - protein, 117 aa, synthetic construct
  REGION 1..117: note = description of the artificial sequence: the amino acid sequenceof I100S antibody VH
QVQLVQSGAEVKKPGASVKVSCKASGYTFTNHYMHWVRQAPGQGLEWMGIINPISGSTSNAQKFQGRVTMTRDTSTSTVYMELSSLRSEDTAVYYCARDSVDAFDFWGQGTMVTVSS

SEQ ID NO: 10 - protein, 117 aa, synthetic construct
  REGION 1..117: note = description of the artificial sequence: the amino acid sequenceof I100R antibody VH
QVQLVQSGAEVKKPGASVKVSCKASGYTFTNHYMHWVRQAPGQGLEWMGIINPISGSTSNAQKFQGRVTMTRDTSTSTVYMELSSLRSEDTAVYYCARDRVDAFDFWGQGTMVTVSS

SEQ ID NO: 11 - protein, 117 aa, synthetic construct
  REGION 1..117: note = description of the artificial sequence: the amino acid sequenceof I100Q antibody VH
QVQLVQSGAEVKKPGASVKVSCKASGYTFTNHYMHWVRQAPGQGLEWMGIINPISGSTSNAQKFQGRVTMTRDTSTSTVYMELSSLRSEDTAVYYCARDQVDAFDFWGQGTMVTVSS

SEQ ID NO: 12 - protein, 117 aa, synthetic construct
  REGION 1..117: note = description of the artificial sequence: the amino acid sequenceof I100N antibody VH
QVQLVQSGAEVKKPGASVKVSCKASGYTFTNHYMHWVRQAPGQGLEWMGIINPISGSTSNAQKFQGRVTMTRDTSTSTVYMELSSLRSEDTAVYYCARDNVDAFDFWGQGTMVTVSS

SEQ ID NO: 13 - protein, 117 aa, synthetic construct
  REGION 1..117: note = description of the artificial sequence: the amino acid sequenceof I100M antibody VH
QVQLVQSGAEVKKPGASVKVSCKASGYTFTNHYMHWVRQAPGQGLEWMGIINPISGSTSNAQKFQGRVTMTRDTSTSTVYMELSSLRSEDTAVYYCARDMVDAFDFWGQGTMVTVSS

SEQ ID NO: 14 - protein, 117 aa, synthetic construct
  REGION 1..117: note = description of the artificial sequence: the amino acid sequenceof I100K antibody VH
QVQLVQSGAEVKKPGASVKVSCKASGYTFTNHYMHWVRQAPGQGLEWMGIINPISGSTSNAQKFQGRVTMTRDTSTSTVYMELSSLRSEDTAVYYCARDKVDAFDFWGQGTMVTVSS

SEQ ID NO: 15 - protein, 117 aa, synthetic construct
  REGION 1..117: note = description of the artificial sequence: the amino acid sequenceof I100H antibody VH
QVQLVQSGAEVKKPGASVKVSCKASGYTFTNHYMHWVRQAPGQGLEWMGIINPISGSTSNAQKFQGRVTMTRDTSTSTVYMELSSLRSEDTAVYYCARDHVDAFDFWGQGTMVTVSS

SEQ ID NO: 16 - protein, 117 aa, synthetic construct
  REGION 1..117: note = description of the artificial sequence: the amino acid sequence of I100G antibody VH
QVQLVQSGAEVKKPGASVKVSCKASGYTFTNHYMHWVRQAPGQGLEWMGIINPISGSTSNAQKFQGRVTMTRDTSTSTVYMELSSLRSEDTAVYYCARDGVDAFDFWGQGTMVTVSS

SEQ ID NO: 17 - protein, 117 aa, synthetic construct
  REGION 1..117: note = description of the artificial sequence: the amino acid sequenceof I100F antibody VH
QVQLVQSGAEVKKPGASVKVSCKASGYTFTNHYMHWVRQAPGQGLEWMGIINPISGSTSNAQKFQGRVTMTRDTSTSTVYMELSSLRSEDTAVYYCARDFVDAFDFWGQGTMVTVSS

SEQ ID NO: 18 - protein, 117 aa, synthetic construct
  REGION 1..117: note = description of the artificial sequence: the amino acid sequenceof I100E antibody VH
QVQLVQSGAEVKKPGASVKVSCKASGYTFTNHYMHWVRQAPGQGLEWMGIINPISGSTSNAQKFQGRVTMTRDTSTSTVYMELSSLRSEDTAVYYCARDEVDAFDFWGQGTMVTVSS

SEQ ID NO: 19 - protein, 117 aa, synthetic construct
  REGION 1..117: note = description of the artificial sequence: the amino acid sequenceof I100D antibody VH
QVQLVQSGAEVKKPGASVKVSCKASGYTFTNHYMHWVRQAPGQGLEWMGIINPISGSTSNAQKFQGRVTMTRDTSTSTVYMELSSLRSEDTAVYYCARDDVDAFDFWGQGTMVTVSS

SEQ ID NO: 20 - protein, 117 aa, synthetic construct
  REGION 1..117: note = description of the artificial sequence: the amino acid sequenceof D105A antibody VH
QVQLVQSGAEVKKPGASVKVSCKASGYTFTNHYMHWVRQAPGQGLEWMGIINPISGSTSNAQKFQGRVTMTRDTSTSTVYMELSSLRSEDTAVYYCARDIVDAFAFWGQGTMVTVSS

SEQ ID NO: 21 - protein, 117 aa, synthetic construct
  REGION 1..117: note = description of the artificial sequence: the amino acid sequenceof D105E antibody VH
QVQLVQSGAEVKKPGASVKVSCKASGYTFTNHYMHWVRQAPGQGLEWMGIINPISGSTSNAQKFQGRVTMTRDTSTSTVYMELSSLRSEDTAVYYCARDIVDAFEFWGQGTMVTVSS

SEQ ID NO: 22 - protein, 117 aa, synthetic construct
  REGION 1..117: note = description of the artificial sequence: the amino acid sequenceof D105F antibody VH
QVQLVQSGAEVKKPGASVKVSCKASGYTFTNHYMHWVRQAPGQGLEWMGIINPISGSTSNAQKFQGRVTMTRDTSTSTVYMELSSLRSEDTAVYYCARDIVDAFFFWGQGTMVTVSS

SEQ ID NO: 23 - protein, 117 aa, synthetic construct
  REGION 1..117: note = description of the artificial sequence: the amino acid sequenceof D105G antibody VH
QVQLVQSGAEVKKPGASVKVSCKASGYTFTNHYMHWVRQAPGQGLEWMGIINPISGSTSNAQKFQGRVTMTRDTSTSTVYMELSSLRSEDTAVYYCARDIVDAFGFWGQGTMVTVSS

SEQ ID NO: 24 - protein, 117 aa, synthetic construct
  REGION 1..117: note = description of the artificial sequence: the amino acid sequenceof D105H antibody VH
QVQLVQSGAEVKKPGASVKVSCKASGYTFTNHYMHWVRQAPGQGLEWMGIINPISGSTSNAQKFQGRVTMTRDTSTSTVYMELSSLRSEDTAVYYCARDIVDAFHFWGQGTMVTVSS

SEQ ID NO: 25 - protein, 117 aa, synthetic construct
  REGION 1..117: note = description of the artificial sequence: the amino acid sequenceof D105I antibody VH
QVQLVQSGAEVKKPGASVKVSCKASGYTFTNHYMHWVRQAPGQGLEWMGIINPISGSTSNAQKFQGRVTMTRDTSTSTVYMELSSLRSEDTAVYYCARDIVDAFIFWGQGTMVTVSS

SEQ ID NO: 26 - protein, 117 aa, synthetic construct
  REGION 1..117: note = description of the artificial sequence: the amino acid sequenceof D105K antibody VH
QVQLVQSGAEVKKPGASVKVSCKASGYTFTNHYMHWVRQAPGQGLEWMGIINPISGSTSNAQKFQGRVTMTRDTSTSTVYMELSSLRSEDTAVYYCARDIVDAFKFWGQGTMVTVSS

SEQ ID NO: 27 - protein, 117 aa, synthetic construct
  REGION 1..117: note = description of the artificial sequence: the amino acid sequenceof D105L antibody VH
QVQLVQSGAEVKKPGASVKVSCKASGYTFTNHYMHWVRQAPGQGLEWMGIINPISGSTSNAQKFQGRVTMTRDTSTSTVYMELSSLRSEDTAVYYCARDIVDAFLFWGQGTMVTVSS

SEQ ID NO: 28 - protein, 117 aa, synthetic construct
  REGION 1..117: note = description of the artificial sequence: the amino acid sequenceof D105M antibody VH
QVQLVQSGAEVKKPGASVKVSCKASGYTFTNHYMHWVRQAPGQGLEWMGIINPISGSTSNAQKFQGRVTMTRDTSTSTVYMELSSLRSEDTAVYYCARDIVDAFMFWGQGTMVTVSS

SEQ ID NO: 29 - protein, 117 aa, synthetic construct
  REGION 1..117: note = description of the artificial sequence: the amino acid sequenceof D105P antibody VH
QVQLVQSGAEVKKPGASVKVSCKASGYTFTNHYMHWVRQAPGQGLEWMGIINPISGSTSNAQKFQGRVTMTRDTSTSTVYMELSSLRSEDTAVYYCARDIVDAFPFWGQGTMVTVSS

SEQ ID NO: 30 - protein, 117 aa, synthetic construct
  REGION 1..117: note = description of the artificial sequence: the amino acid sequenceof D105Q antibody VH
QVQLVQSGAEVKKPGASVKVSCKASGYTFTNHYMHWVRQAPGQGLEWMGIINPISGSTSNAQKFQGRVTMTRDTSTSTVYMELSSLRSEDTAVYYCARDIVDAFQFWGQGTMVTVSS

SEQ ID NO: 31 - protein, 117 aa, synthetic construct
  REGION 1..117: note = description of the artificial sequence: the amino acid sequenceof D105R antibody VH
QVQLVQSGAEVKKPGASVKVSCKASGYTFTNHYMHWVRQAPGQGLEWMGIINPISGSTSNAQKFQGRVTMTRDTSTSTVYMELSSLRSEDTAVYYCARDIVDAFRFWGQGTMVTVSS

SEQ ID NO: 32 - protein, 117 aa, synthetic construct
  REGION 1..117: note = description of the artificial sequence: the amino acid sequenceof D105V antibody VH
QVQLVQSGAEVKKPGASVKVSCKASGYTFTNHYMHWVRQAPGQGLEWMGIINPISGSTSNAQKFQGRVTMTRDTSTSTVYMELSSLRSEDTAVYYCARDIVDAFVFWGQGTMVTVSS

SEQ ID NO: 33 - protein, 117 aa, synthetic construct
  REGION 1..117: note = description of the artificial sequence: the amino acid sequenceof D105W antibody VH
QVQLVQSGAEVKKPGASVKVSCKASGYTFTNHYMHWVRQAPGQGLEWMGIINPISGSTSNAQKFQGRVTMTRDTSTSTVYMELSSLRSEDTAVYYCARDIVDAFWFWGQGTMVTVSS

SEQ ID NO: 34 - protein, 117 aa, synthetic construct
  REGION 1..117: note = description of the artificial sequence: the amino acid sequenceof D105Y antibody VH
QVQLVQSGAEVKKPGASVKVSCKASGYTFTNHYMHWVRQAPGQGLEWMGIINPISGSTSNAQKFQGRVTMTRDTSTSTVYMELSSLRSEDTAVYYCARDIVDAFYFWGQGTMVTVSS

SEQ ID NO: 35 - protein, 117 aa, synthetic construct
  REGION 1..117: note = description of the artificial sequence: the amino acid sequenceof D105T antibody VH
QVQLVQSGAEVKKPGASVKVSCKASGYTFTNHYMHWVRQAPGQGLEWMGIINPISGSTSNAQKFQGRVTMTRDTSTSTVYMELSSLRSEDTAVYYCARDIVDAFTFWGQGTMVTVSS

SEQ ID NO: 36 - protein, 117 aa, synthetic construct
  REGION 1..117: note = description of the artificial sequence: the amino acid sequenceof D105N antibody VH
QVQLVQSGAEVKKPGASVKVSCKASGYTFTNHYMHWVRQAPGQGLEWMGIINPISGSTSNAQKFQGRVTMTRDTSTSTVYMELSSLRSEDTAVYYCARDIVDAFNFWGQGTMVTVSS

SEQ ID NO: 37 - protein, 117 aa, synthetic construct
  REGION 1..117: note = description of the artificial sequence: the amino acid sequenceof D105Santibody VH
QVQLVQSGAEVKKPGASVKVSCKASGYTFTNHYMHWVRQAPGQGLEWMGIINPISGSTSNAQKFQGRVTMTRDTSTSTVYMELSSLRSEDTAVYYCARDIVDAFSFWGQGTMVTVSS

SEQ ID NO: 38 - protein, 117 aa, synthetic construct
  REGION 1..117: note = description of the artificial sequence: the amino acid sequenceof H2B11_A
QVQLVQSGAEVKKPGASVKVSCKASGYTFTNHYMHWVRQAPGQGLEWMGIVNPFWGRWSNAQKFQGRVTMTRDTSTSTVYMELSSLRSEDTAVYYCARDAVDAFDFWGQGTMVTVSS

SEQ ID NO: 39 - protein, 117 aa, synthetic construct
  REGION 1..117: note = description of the artificial sequence: the amino acid sequenceof J2H2B9_A
QVQLVQSGAEVKKPGASVKVSCKASGYTFTNHYMHWVRQAPGQGLEWMGLINPWHGTFSNAQKFQGRVTMTRDTSTSTVYMELSSLRSEDTAVYYCARDAVDAFDFWGQGTMVTVSS

SEQ ID NO: 40 - protein, 117 aa, synthetic construct
  REGION 1..117: note = description of the artificial sequence: the amino acid sequenceof J2H2E9_A
QVQLVQSGAEVKKPGASVKVSCKASGYTFTNHYMHWVRQAPGQGLEWMGVINPFCGFVSNAQKFQGRVTMTRDTSTSTVYMELSSLRSEDTAVYYCARDAVDAFDFWGQGTMVTVSS

SEQ ID NO: 41 - protein, 117 aa, synthetic construct
  REGION 1..117: note = description of the artificial sequence: the amino acid sequenceof 2H2E1_A
QVQLVQSGAEVKKPGASVKVSCKASGYTFTNHYMHWVRQAPGQGLEWMGILNPWTGYRSNAQKFQGRVTMTRDTSTSTVYMELSSLRSEDTAVYYCARDAVDAFDFWGQGTMVTVSS

SEQ ID NO: 42 - protein, 117 aa, synthetic construct
  REGION 1..117: note = description of the artificial sequence: the amino acid sequenceof 2H2E5_A
QVQLVQSGAEVKKPGASVKVSCKASGYTFTNHYMHWVRQAPGQGLEWMGIINPWVGRASNAQKFQGRVTMTRDTSTSTVYMELSSLRSEDTAVYYCARDAVDAFDFWGQGTMVTVSS

SEQ ID NO: 43 - protein, 117 aa, synthetic construct
  REGION 1..117: note = description of the artificial sequence: the amino acid sequenceof 2H2E8_Y
QVQLVQSGAEVKKPGASVKVSCKASGYTFTNHYMHWVRQAPGQGLEWMGIVNPYRGKWSNAQKFQGRVTMTRDTSTSTVYMELSSLRSEDTAVYYCARDYVDAFDFWGQGTMVTVSS

SEQ ID NO: 44 - protein, 106 aa, synthetic construct
  REGION 1..106: note = description of the artificial sequence: the amino acid sequenceof L3G12
AIQLTQSPSSLSASVGDRVTITCRASQGISSALVWYQQKPGKAPKLLIYDASSLESGVPSRFSGSGSGTDFTLTISSLQPEDFATYYCQQMYDDFNFGPGTKVDIK

SEQ ID NO: 45 - protein, 106 aa, synthetic construct
  REGION 1..106: note = description of the artificial sequence: the amino acid sequenceof L1H8
AIQLTQSPSSLSASVGDRVTITCRASQDVSTALLWYQQKPGKAPKLLIYDASSLESGVPSRFSGSGSGTDFTLTISSLQPEDFATYYCQQFNDYFTFGPGTKVDIK

SEQ ID NO: 46 - protein, 106 aa, synthetic construct
  REGION 1..106: note = description of the artificial sequence: the amino acid sequenceof 2L3H7
AIQLTQSPSSLSASVGDRVTITCRASQGISSALVWYQQKPGKAPKLLIYDASSLESGVPSRFSGSGSGTDFTLTISSLQPEDFATYYCQQLYDDFDFGPGTKVDIK

SEQ ID NO: 47 - protein, 117 aa, synthetic construct
  REGION 1..117: note = description of the artificial sequence: the amino acid sequenceof J2H2B9_Y
QVQLVQSGAEVKKPGASVKVSCKASGYTFTNHYMHWVRQAPGQGLEWMGLINPWHGTFSNAQKFQGRVTMTRDTSTSTVYMELSSLRSEDTAVYYCARDYVDAFDFWGQGTMVTVSS

SEQ ID NO: 48 - protein, 330 aa, synthetic construct
  REGION 1..330: note = description of the artificial sequence: the amino acid sequenceof YTE CH
ASTKGPSVFPLAPSSKSTSGGTAALGCLVKDYFPEPVTVSWNSGALTSGVHTFPAVLQSSGLYSLSSVVTVPSSSLGTQTYICNVNHKPSNTKVDKKVEPKSCDKTHTCPPCPAPELLGGPSVFLFPPKPKDTLYITREPEVTCVVVDVSHEDPEVKFNWYVDGVEVHNAKTKPREEQYNSTYRVVSVLTVLHQDWLNGKEYKCKVSNKALPAPIEKTISKAKGQPREPQVYTLPPSRDELTKNQVSLTCLVKGFYPSDIAVEWESNGQPENNYKTTPPVLDSDGSFFLYSKLTVDKSRWQQGNVFSCSVMHEALHNHYTQKSLSLSPGK

SEQ ID NO: 49 - protein, 326 aa, synthetic construct
  REGION 1..326: note = description of the artificial sequence: the amino acid sequenceof G2_YTE CH
ASTKGPSVFPLAPCSRSTSESTAALGCLVKDYFPEPVTVSWNSGALTSGVHTFPAVLQSSGLYSLSSVVTVPSSNFGTQTYTCNVDHKPSNTKVDKTVERKCCVECPPCPAPPVAGPSVFLFPPKPKDTLYITREPEVTCVVVDVSHEDPEVQFNWYVDGVEVHNAKTKPREEQFNSTFRVVSVLTVVHQDWLNGKEYKCKVSNKGLPAPIEKTISKTKGQPREPQVYTLPPSREEMTKNQVSLTCLVKGFYPSDIAVEWESNGQPENNYKTTPPMLDSDGSFFLYSKLTVDKSRWQQGNVFSCSVMHEALHNHYTQKSLSLSPGK

SEQ ID NO: 50 - protein, 326 aa, synthetic construct
  REGION 1..326: note = description of the artificial sequence: the amino acid sequenceof G2_LS CH
ASTKGPSVFPLAPCSRSTSESTAALGCLVKDYFPEPVTVSWNSGALTSGVHTFPAVLQSSGLYSLSSVVTVPSSNFGTQTYTCNVDHKPSNTKVDKTVERKCCVECPPCPAPPVAGPSVFLFPPKPKDTLMISRTPEVTCVVVDVSHEDPEVQFNWYVDGVEVHNAKTKPREEQFNSTFRVVSVLTVVHQDWLNGKEYKCKVSNKGLPAPIEKTISKTKGQPREPQVYTLPPSREEMTKNQVSLTCLVKGFYPSDIAVEWESNGQPENNYKTTPPMLDSDGSFFLYSKLTVDKSRWQQGNVFSCSVLHEALHSHYTQKSLSLSPGK

SEQ ID NO: 51 - protein, 327 aa, synthetic construct
  REGION 1..327: note = description of the artificial sequence: the amino acid sequenceof G4PE_R409K_P CH
ASTKGPSVFPLAPCSRSTSESTAALGCLVKDYFPEPVTVSWNSGALTSGVHTFPAVLQSSGLYSLSSVVTVPSSSLGTKTYTCNVDHKPSNTKVDKRVESKYGPPCPPCPAPEFEGGPSVFLFPPKPKDTLMISRTPEVTCVVVDVSQEDPEVQFNWYVDGVEVHNAKTKPREEQFNSTYRVVSVLTPLHQDWLNGKEYKCKVSNKGLPSSIEKTISKAKGQPREPQVYTLPPSQEEMTKNQVSLTCLVKGFYPSDIAVEWESNGQPENNYKTTPPVLDSDGSFFLYSKLTVDKSRWQEGNVFSCSVMHEALHNHYTQKSLSLSLGK

SEQ ID NO: 52 - protein, 327 aa, synthetic construct
  REGION 1..327: note = description of the artificial sequence: the amino acid sequenceof G4PE_R409K_LS CH
ASTKGPSVFPLAPCSRSTSESTAALGCLVKDYFPEPVTVSWNSGALTSGVHTFPAVLQSSGLYSLSSVVTVPSSSLGTKTYTCNVDHKPSNTKVDKRVESKYGPPCPPCPAPEFEGGPSVFLFPPKPKDTLMISRTPEVTCVVVDVSQEDPEVQFNWYVDGVEVHNAKTKPREEQFNSTYRVVSVLTVLHQDWLNGKEYKCKVSNKGLPSSIEKTISKAKGQPREPQVYTLPPSQEEMTKNQVSLTCLVKGFYPSDIAVEWESNGQPENNYKTTPPVLDSDGSFFLYSKLTVDKSRWQEGNVFSCSVLHEALHSHYTQKSLSLSLGK

SEQ ID NO: 53 - protein, 330 aa, synthetic construct [sequence omitted]

SEQ ID NO: 54 - protein, 303 aa, synthetic construct
  REGION 1..303: note = description of the artificial sequence: the amino acid sequenceof Homo sapiens FcRn extracellular domain His-tag form
MGVPRPQPWALGLLLFLLPGSLGAESHLSLLYHLTAVSSPAPGTPAFWVSGWLGPQQYLSYNSLRGEAEPCGAWVWENQVSWYWEKETTDLRIKEKLFLEAFKALGGKGPYTLQGLLGCELGPDNTSVPTAKFALNGEEFMNFDLKQGTWGGDWPEALAISQRWQQQDKAANKELTFLLFSCPHRLREHLERGRGNLEWKEPPSMRLKARPSSPGFSVLTCSAFSFYPPELQLRFLRNGLAAGTGQGDFGPNSDGSFHASSSLTVKSGDEHHYCCIVQHAGLAQPLRVELESPAKSSHHHHHH

SEQ ID NO: 55 - protein, 119 aa, Homo sapiens
MSRSVALAVLALLSLSGLEAIQRTPKIQVYSRHPAENGKSNFLNCYVSGFHPSDIEVDLLKNGERIEKVEHSDLSFSKDWSFYLLYYTEFTPTEKDEYACRVNHVTLSQPKIVKWDRDM

SEQ ID NO: 56 - protein, 303 aa, synthetic construct
  REGION 1..303: note = description of the artificial sequence: the amino acid sequenceof Primates FcRn extracellular domain His-tag form
MRVPRPQPWALGLLLFLLPGSLGAESHLSLLYHLTAVSSPAPGTPAFWVSGWLGPQQYLSYDSLRGQAEPCGAWVWENQVSWYWEKETTDLRIKEKLFLEAFKALGGKGPYTLQGLLGCELSPDNTSVPTAKFALNGEEFMNFDLKQGTWGGDWPEALAISQRWQQQDKAANKELTFLLFSCPHRLREHLERGRGNLEWKEPPSMRLKARPGNPGFSVLTCSAFSFYPPELQLRFLRNGMAAGTGQGDFGPNSDGSFHASSSLTVKSGDEHHYCCIVQHAGLAQPLRVELETPAKSSHHHHHH

SEQ ID NO: 57 - protein, 119 aa, Primates
MSPSVALAVLALLSPSGLEAIQRTPKIQVYSRHPPENGKPNFLNCYVSGFHPSDIEVDLLKNGEKMGKVEHSDLSFSKDWSFYLLYYTEFTPNEKDEYACRVNHVTLSGPRTVKWDRDM

SEQ ID NO: 58 - protein, 106 aa, synthetic construct
  REGION 1..106: note = description of the artificial sequence: the amino acid sequence of A-9 antibody VL
AIQLTQSPSSLSASVGDRVTITCRASQGISSALVWYQQKPGKAPKLLIYDASSLESGVPSRFSGSGSGTDFTLTISSLQPEDFATYYCQQFWDDFDFGPGTKVDIK

SEQ ID NO: 59 - protein, 106 aa, synthetic construct
  REGION 1..106: note = description of the artificial sequence: the amino acid sequence of A-10 antibody VL
AIQLTQSPSSLSASVGDRVTITCRASQGISSALVWYQQKPGKAPKLLIYDASSLESGVPSRFSGSGSGTDFTLTISSLQPEDFATYYCQQFYDDFDFGPGTKVDIK